European Patent Specification EP 3 402 822 B1, published March 12, 2025. Title: AXL-SPECIFIC ANTIBODY-DRUG CONJUGATES FOR CANCER TREATMENT. Applicant: Genmab A/S. The sequence listing filed with the application follows.

SEQUENCE LISTING (153 sequences)

SEQ ID NO: 1 - protein, 116 aa, homo sapiens
EVQLLESGGGLVQPGGSLRLSCAASGFTFSSYAMNWVRQAPGKGLEWVSTTSGSGASTYYADSVKGRFTISRDNSKNTLYLQMNSLRAEDTAVYYCAKIWIAFDIWGQGTMVTVSS

SEQ ID NO: 2 - protein, 108 aa, homo sapiens
EIVLTQSPGTLSLSPGERATLSCRASQSVSSSYLAWYQQKPGQAPRLLIYGASSRATGIPDRFSGSGSGTDFTLTISRLEPEDFAVYYCQQYGSSPYTFGQGTKLEIK

SEQ ID NO: 3 - protein, 120 aa, homo sapiens
EVQLLESGGGLVQPGGSLRLSCAASGFTFSSYAMTWVRQAPGKGLEWVSAISISGASTFYADSVKGRFTISRDNSKNTLSLQMNSLRAEDTAVYFCRGYSGYVYDAFDIWGQGTMVTVSS

SEQ ID NO: 4 - protein, 107 aa, homo sapiens
DIQMTQSPSSLSASVGDRVTITCRASQGISNWLAWYQQKPEKAPKSLIYAASSLQSGVPSRFSGSGSGTDFTLTISSLQPEDFATYYCQQYNSYPLTFGGGTKVEIK

SEQ ID NO: 5 - protein, 120 aa, homo sapiens
EVQLLESGGGLVQPGGSLRLSCAASGFTFSSYAMTWVRQAPGKGLEWVSAISISGGSTFYADSVKGRFTISRDNSKNTLYLQMNSLRAEDTAVYYCRGYSGYVYDAFDFWGQGTMVTVSS

SEQ ID NO: 6 - protein, 107 aa, homo sapiens; identical to SEQ ID NO: 4

SEQ ID NO: 7 - protein, 121 aa, homo sapiens
EVQLLDSGGGLVQPGGSLRLSCAASGFTFSSYAMSWVRQAPGKGLEWVSAISIGGGNAYYADSVKGRFTISRDNSKNTLYLQMNSLRAADTAVYYCAKPGFIMVRGPLDYWGQGALVTVSS

SEQ ID NO: 8 - protein, 121 aa, homo sapiens
EVQLLDSGGGLVQPGGSLRLSCAASGFTFSSYAMSWVRQAPGKGLEWVSAISIGGGNAYYADSVKGRFTISRDNSKNTLYLQMNSLRAADTAVYYCAKPGFILVRGPLDYWGQGALVTVSS

SEQ ID NO: 9 - protein, 108 aa, homo sapiens
EIVLTQSPGTLSLSPGERATLSCRASQSVSNSYLAWYQQKPGQAPRLLIYGASSRATGIPDRFSGSGSGTDFTLTISRLEPEDFAVYYCQQYGSSPYTFGQGTKLEIK

SEQ ID NO: 10 - protein, 125 aa, homo sapiens
EVQLLESGGGLVQPGGSLRLSCAASGFTFSSYAMSWVRQAPGKGLEWVSDISVSGGSTYYADSVKGRFTISRDNSKNTLYLQMNSLRAEDTAVYYCAKEGYIWFGESLSYAFDIWGQGTMVTVSS

SEQ ID NO: 11 - protein, 107 aa, homo sapiens
EIVLTQSPGTLSLSPGERATLSCRASQSVSSSYLAWYQQKPGQAPRLLIYGASSRATGIPDRFSGSGSGTDFTLTISRLEPEDFAVYYCQQYGRSFTFGPGTKVDIK

SEQ ID NO: 12 - protein, 125 aa, homo sapiens
EVQLLESGGGLVQPGGSLRLSCAASGFTFSNYAMSWVRQAPGKGLEWVSDISVSGGSTYYADSVKGRFTISRDNSKNTLYLQMNSLRAEDTAVYYCAKEGYIWFGESLSYAFDIWGQGTMVTVSS

SEQ ID NO: 13 - protein, 107 aa, homo sapiens; identical to SEQ ID NO: 11

SEQ ID NO: 14 - protein, 125 aa, homo sapiens
EVQLLESGGGLVQPGGSLRLSCAASGFTFSSYAMSWVRQAPGKGLEWVSDISVSGGSTYYADSVKGRFTISRDNSKNTLYLHMNSLRAEDTAVYYCAKEGYIWFGESLSYAFDIWGQGTMVTVSS

SEQ ID NO: 15 - protein, 107 aa, homo sapiens; identical to SEQ ID NO: 11

SEQ ID NO: 16 - protein, 117 aa, homo sapiens
QVQLQQWGAGLLKPSETLSLTCAVYGGSFSGYYWSWIRQPPGKGLEWIGEINQSGSTNYNPSLKSRVTISVDTSKNQFSLKLSSVTAADTSVYYCASGNWDHFFDYWGQGTLVTVSS

SEQ ID NO: 17 - protein, 117 aa, homo sapiens
QVQLQQWGAGLLKPSETLSLTCAVYGGSFSGYYWSWIRQPPGKGLEWIGEIQQSGSTNYNPSLKSRVTISVDTSKNQFSLKLSSVTAADTSVYYCASGNWDHFFDYWGQGTLVTVSS

SEQ ID NO: 18 - protein, 107 aa, homo sapiens
DIQMTQSPSSVSASVGDRVTITCRASQGISSWLAWYQHKPGKAPKLLIYATSSLQSGVTSRFSGSGSGTDFTLTISSLQPEDFATYYCQQAKSFPWTFGQGTKVEIK

SEQ ID NO: 19 - protein, 123 aa, homo sapiens
QVPLQQWGAGLLKPSETLSLTCAVYGGSFSGYHWSWIRQPPGKGLEWIGEISHSGRTNYNPSLKSRVTISIDTSKNQFSLKLSSVTAADTAVYYCASFITMIRGTIITHFDYWGQGTLVTVSS

SEQ ID NO: 20 - protein, 107 aa, homo sapiens
DIQMTQSPSSLSASVGDRVTITCRASQGISSWLAWYQQKPEKAPKSLIYAASSLQSGVPSRFSGSGSGTDFTLTISSLQPEDFATYYCQQYHSYPYTFGQGTKLEIK

SEQ ID NO: 21 - protein, 124 aa, homo sapiens
QVQLVQSGAEVKKPGSSVKVSCKASGGTFSSYAISWVRQAPGQGLEWMGRIIPIFGIANYVQKFQGRVTITADKSTSTAYMELSSLRAEDTAVYYCARRGDYYGSGSPDVFDIWGQGTMVTVSS

SEQ ID NO: 22 - protein, 107 aa, homo sapiens
EIVLTQSPGTLSLSPGERATLSCRASQSVSSSYLAWYQQKPGQAPRLLIYGASSRATGIPDRFSGSGSGTDFTLTISRLEPEDFAVYYCQQYGSSYTFGQGTKLEIK

SEQ ID NO: 23 - protein, 124 aa, homo sapiens
QVQLVQSGAEVKKPGSSVKVSCKASGGTFSSYAISWVRQAPGQGLEWMGRIIPIFGIANYVQKFQGRVTITADKSTSTAYMELSSLRAEDTAVYYCARRGNYYGSGSPDVFDIWGQGTMVTVSS

SEQ ID NO: 24 - protein, 107 aa, homo sapiens; identical to SEQ ID NO: 22

SEQ ID NO: 25 - protein, 124 aa, homo sapiens
QVQLVQSGAEVKKPGSSVKVSCKASGGTFSSYAINWMRQAPGQGLEWMGRIIPIFGIVNYAQKFQGRVTLTADKSTSTAYMELSSLRSEDTAVYYCARRGNYYGSGSPDVFDIWGQGTMVTVSS

SEQ ID NO: 26 - protein, 107 aa, homo sapiens; identical to SEQ ID NO: 22

SEQ ID NO: 27 - protein, 124 aa, homo sapiens; identical to SEQ ID NO: 25

SEQ ID NO: 28 - protein, 106 aa, homo sapiens
EIVLTQSPATLSLSPGERATLSCRASQSVSSYLAWYQQKPGQAPRLLIYDASNRATGIPARFSGSGSGTDFTLTISSLEPEDFAVYYCQQRSNWLTFGGGTKVEIK

SEQ ID NO: 29 - protein, 124 aa, homo sapiens
QVQLVQSGAEVKKPGSSVKVSCKASGGTFSSYAISWVRQAPGQGLEWMGRIIPIFGIANYAQKFQGRVTITADKSTSTAYMELSSLRSEDTAVYYCARRGNYYGSGSPDVFDIWGQGTMVTVSS

SEQ ID NO: 30 - protein, 107 aa, homo sapiens; identical to SEQ ID NO: 22

SEQ ID NO: 31 - protein, 123 aa, homo sapiens
QVQLQQWGAGLLKPSETLSLTCAIDGGSFSGYYWSWIRQPPGKGLEWIGEISHSGRTNYNPSLKSRVTISIDTSKNQFSLKLSSVAAADTAVYYCARFITMIRGAIITHFDYWGQGALVTVSS

SEQ ID NO: 32 - protein, 123 aa, homo sapiens
QVQLQQWGAGLLKPSETLSLTCAIDGGSFSGYYWSWIRQPPGKGLEWIGEISHSGRTNYNPSLKSRVTISIDTSKNQFSLKLSSVAAADTAVYYCARFITLIRGAIITHFDYWGQGALVTVSS

SEQ ID NO: 33 - protein, 107 aa, homo sapiens; identical to SEQ ID NO: 20

SEQ ID NO: 34 - protein, 120 aa, homo sapiens
QVQLVESGGGVVQPGRSLRLSCAASGFSFSTYAMHWVRQAPGKGLEWVAVISYDGDNKYSADSVKGRFTISRDNSKNTLYLQMNSLRAEDTAVYYCARGRKLGIDAFDIWGQGTMVTVSS

SEQ ID NO: 35 - protein, 107 aa, homo sapiens
AIQLTQSPSSLSASVGDRVTITCRASQGISSALAWYQQKPGKAPKLLIYDASSLESGVPSRFSGSGSGTDFTLTISGLQPEDFATYYCQQFNSYPFTFGPGTKVDIK

SEQ ID NO: 36 - protein, 8 aa, homo sapiens
GFTFSSYA

SEQ ID NO: 37 - protein, 8 aa, homo sapiens
TSGSGAST

SEQ ID NO: 38 - protein, 9 aa, homo sapiens
AKIWIAFDI

SEQ ID NO: 39 - protein, 7 aa, homo sapiens
QSVSSSY

SEQ ID NO: 40 - protein, 9 aa, homo sapiens
QQYGSSPYT

SEQ ID NO: 41 - protein, 8 aa, homo sapiens
GFTFSSYA

SEQ ID NO: 42 - protein, 8 aa, homo sapiens
ISISGAST

SEQ ID NO: 43 - protein, 13 aa, homo sapiens
RGYSGYVYDAFDI

SEQ ID NO: 44 - protein, 6 aa, homo sapiens
QGISNW

SEQ ID NO: 45 - protein, 9 aa, homo sapiens
QQYNSYPLT

SEQ ID NO: 46 - protein, 8 aa, homo sapiens
GFTFSSYA

SEQ ID NO: 47 - protein, 8 aa, homo sapiens
ISISGGST

SEQ ID NO: 48 - protein, 13 aa, homo sapiens
RGYSGYVYDAFDF

SEQ ID NO: 49 - protein, 6 aa, homo sapiens
QGISNW

SEQ ID NO: 50 - protein, 9 aa, homo sapiens
QQYNSYPLT

SEQ ID NO: 51 - protein, 8 aa, homo sapiens
GFTFSSYA

SEQ ID NO: 52 - protein, 8 aa, homo sapiens
ISIGGGNA

SEQ ID NO: 53 - protein, 14 aa, homo sapiens
AKPGFIMVRGPLDY

SEQ ID NO: 54 - protein, 14 aa, homo sapiens
AKPGFILVRGPLDY

SEQ ID NO: 55 - protein, 7 aa, homo sapiens
QSVSNSY

SEQ ID NO: 56 - protein, 9 aa, homo sapiens
QQYGSSPYT

SEQ ID NO: 57 - protein, 8 aa, homo sapiens
GFTFSSYA

SEQ ID NO: 58 - protein, 8 aa, homo sapiens
ISVSGGST

SEQ ID NO: 59 - protein, 18 aa, homo sapiens
AKEGYIWFGESLSYAFDI

SEQ ID NO: 60 - protein, 7 aa, homo sapiens
QSVSSSY

SEQ ID NO: 61 - protein, 8 aa, homo sapiens
QQYGRSFT

SEQ ID NO: 62 - protein, 8 aa, homo sapiens
GFTFSNYA

SEQ ID NO: 63 - protein, 8 aa, homo sapiens
ISVSGGST

SEQ ID NO: 64 - protein, 18 aa, homo sapiens
AKEGYIWFGESLSYAFDI

SEQ ID NO: 65 - protein, 7 aa, homo sapiens
QSVSSSY

SEQ ID NO: 66 - protein, 8 aa, homo sapiens
QQYGRSFT

SEQ ID NO: 67 - protein, 8 aa, homo sapiens
GFTFSSYA

SEQ ID NO: 68 - protein, 8 aa, homo sapiens
ISVSGGST

SEQ ID NO: 69 - protein, 18 aa, homo sapiens
AKEGYIWFGESLSYAFDI

SEQ ID NO: 70 - protein, 7 aa, homo sapiens
QSVSSSY

SEQ ID NO: 71 - protein, 8 aa, homo sapiens
QQYGRSFT

SEQ ID NO: 72 - protein, 8 aa, homo sapiens
GGSFSGYY

SEQ ID NO: 73 - protein, 5 aa, homo sapiens
INQSG

SEQ ID NO: 74 - protein, 7 aa, homo sapiens
IQQSGST

SEQ ID NO: 75 - protein, 11 aa, homo sapiens
ASGNWDHFFDY

SEQ ID NO: 76 - protein, 6 aa, homo sapiens
QGISSW

SEQ ID NO: 77 - protein, 9 aa, homo sapiens
QQAKSFPWT

SEQ ID NO: 78 - protein, 8 aa, homo sapiens
GGSFSGYH

SEQ ID NO: 79 - protein, 7 aa, homo sapiens
ISHSGRT

SEQ ID NO: 80 - protein, 17 aa, homo sapiens
ASFITMIRGTIITHFDY

SEQ ID NO: 81 - protein, 6 aa, homo sapiens
QGISSW

SEQ ID NO: 82 - protein, 9 aa, homo sapiens
QQYHSYPYT

SEQ ID NO: 83 - protein, 8 aa, homo sapiens
GGTFSSYA

SEQ ID NO: 84 - protein, 8 aa, homo sapiens
IIPIFGIA

SEQ ID NO: 85 - protein, 17 aa, homo sapiens
ARRGDYYGSGSPDVFDI

SEQ ID NO: 86 - protein, 7 aa, homo sapiens
QSVSSSY

SEQ ID NO: 87 - protein, 8 aa, homo sapiens
QQYGSSYT

SEQ ID NO: 88 - protein, 8 aa, homo sapiens
GGTFSSYA

SEQ ID NO: 89 - protein, 8 aa, homo sapiens
IIPIFGIA

SEQ ID NO: 90 - protein, 17 aa, homo sapiens
ARRGNYYGSGSPDVFDI

SEQ ID NO: 91 - protein, 7 aa, homo sapiens
QSVSSSY

SEQ ID NO: 92 - protein, 8 aa, homo sapiens
QQYGSSYT

SEQ ID NO: 93 - protein, 8 aa, homo sapiens
GGTFSSYA

SEQ ID NO: 94 - protein, 8 aa, homo sapiens
IIPIFGIV

SEQ ID NO: 95 - protein, 17 aa, homo sapiens
ARRGNYYGSGSPDVFDI

SEQ ID NO: 96 - protein, 7 aa, homo sapiens
QSVSSSY

SEQ ID NO: 97 - protein, 8 aa, homo sapiens
QQYGSSYT

SEQ ID NO: 98 - protein, 8 aa, homo sapiens
GGTFSSYA

SEQ ID NO: 99 - protein, 8 aa, homo sapiens
IIPIFGIV

SEQ ID NO: 100 - protein, 17 aa, homo sapiens
ARRGNYYGSGSPDVFDI

SEQ ID NO: 101 - protein, 6 aa, homo sapiens
QSVSSY

SEQ ID NO: 102 - protein, 8 aa, homo sapiens
QQRSNWLT

SEQ ID NO: 103 - protein, 8 aa, homo sapiens
GGTFSSYA

SEQ ID NO: 104 - protein, 8 aa, homo sapiens
IIPIFGIA

SEQ ID NO: 105 - protein, 18 aa, homo sapiens
ARRGNYYGSGSPDVFDIS

SEQ ID NO: 106 - protein, 7 aa, homo sapiens
QSVSSSY

SEQ ID NO: 107 - protein, 8 aa, homo sapiens
QQYGSSYT

SEQ ID NO: 108 - protein, 8 aa, homo sapiens
GGSFSGYY

SEQ ID NO: 109 - protein, 7 aa, homo sapiens
ISHSGRT

SEQ ID NO: 110 - protein, 17 aa, homo sapiens
ARFITMIRGAIITHFDY

SEQ ID NO: 111 - protein, 17 aa, homo sapiens
ARFITLIRGAIITHFDY

SEQ ID NO: 112 - protein, 6 aa, homo sapiens
QGISSW

SEQ ID NO: 113 - protein, 9 aa, homo sapiens
QQYHSYPYT

SEQ ID NO: 114 - protein, 8 aa, homo sapiens
GFSFSTYA

SEQ ID NO: 115 - protein, 8 aa, homo sapiens
ISYDGDNK

SEQ ID NO: 116 - protein, 13 aa, homo sapiens
ARGRKLGIDAFDI

SEQ ID NO: 117 - protein, 6 aa, homo sapiens
QGISSA

SEQ ID NO: 118 - protein, 9 aa, homo sapiens
QQFNSYPFT

SEQ ID NO: 119 - protein, 8 aa, homo sapiens
  MISC_FEATURE (6)..(6): Wherein X is A or G
ISISGXST

SEQ ID NO: 120 - protein, 13 aa, homo sapiens
  Misc (13)..(13): Wherein X is I of F
RGYSGYVYDAFDX

SEQ ID NO: 121 - protein, 8 aa, homo sapiens
  MISC_FEATURE (8)..(8): Wherein X is I or F
GGSFSGYX

SEQ ID NO: 122 - protein, 17 aa, homo sapiens
  MISC_FEATURE (2)..(2): Wherein X is S or R
  MISC_FEATURE (10)..(10): Wherein X is T or A
AXFITMIRGXIITHFDY

SEQ ID NO: 123 - protein, 8 aa, homo sapiens
  MISC_FEATURE (6)..(6): Wherein X is S or N
GFTFSXYA

SEQ ID NO: 124 - protein, 8 aa, homo sapiens
ISVSGGST

SEQ ID NO: 125 - protein, 18 aa, homo sapiens
AKEGYIWFGESLSYAFDI

SEQ ID NO: 126 - protein, 8 aa, homo sapiens
  MISC_FEATURE (8)..(8): Wherein X is A or V
IIPIFGIX

SEQ ID NO: 127 - protein, 17 aa, homo sapiens
  MISC_FEATURE (5)..(5): Wherein X is D or N
ARRGXYYGSGSPDVFDI

SEQ ID NO: 128 - protein, 7 aa, homo sapiens
  MISC_FEATURE (4)..(4): Wherein X is S or deleted
QSVXSSY

SEQ ID NO: 129 - protein, 8 aa, homo sapiens
  MISC_FEATURE (3)..(3): Wherein X is R or Y
  MISC_FEATURE (4)..(4): Wherein X is Sor G
  MISC_FEATURE (4)..(4): Wherein X is Sor G
  MISC_FEATURE (5)..(5): Wherein X is N or S
  MISC_FEATURE (6)..(6): Wherein X is W or S
  MISC_FEATURE (6)..(6): Wherein X is W or S
  MISC_FEATURE (7)..(7): Wherein X is L or Y
QQXXXXXT

SEQ ID NO: 130 - protein, 894 aa, homo sapiens
MAWRCPRMGRVPLAWCLALCGWACMAPRGTQAEESPFVGNPGNITGARGLTGTLRCQLQVQGEPPEVHWLRDGQILELADSTQTQVPLGEDEQDDWIVVSQLRITSLQLSDTGQYQCLVFLGHQTFVSQPGYVGLEGLPYFLEEPEDRTVAANTPFNLSCQAQGPPEPVDLLWLQDAVPLATAPGHGPQRSLHVPGLNKTSSFSCEAHNAKGVTTSRTATITVLPQQPRNLHLVSRQPTELEVAWTPGLSGIYPLTHCTLQAVLSDDGMGIQAGEPDPPEEPLTSQASVPPHQLRLGSLHPHTPYHIRVACTSSQGPSSWTHWLPVETPEGVPLGPPENISATRNGSQAFVHWQEPRAPLQGTLLGYRLAYQGQDTPEVLMDIGLRQEVTLELQGDGSVSNLTVCVAAYTAAGDGPWSLPVPLEAWRPGQAQPVHQLVKEPSTPAFSWPWWYVLLGAVVAAACVLILALFLVHRRKKETRYGEVFEPTVERGELVVRYRVRKSYSRRTTEATLNSLGISEELKEKLRDVMVDRHKVALGKTLGEGEFGAVMEGQLNQDDSILKVAVKTMKIAICTRSELEDFLSEAVCMKEFDHPNVMRLIGVCFQGSERESFPAPVVILPFMKHGDLHSFLLYSRLGDQPVYLPTQMLVKFMADIASGMEYLSTKRFIHRDLAARNCMLNENMSVCVADFGLSKKIYNGDYYRQGRIAKMPVKWIAIESLADRVYTSKSDVWSFGVTMWEIATRGQTPYPGVENSEIYDYLRQGNRLKQPADCLDGLYALMSRCWELNPQDRPSFTELREDLENTLKALPPAQEPDEILYVNMDEGGGYPEPPGAAGGADPPTQPDPKDSCSCLTAAEVHPAGRYVLCPSTTPSPAQPADRGSPAAPGQEDGA

SEQ ID NO: 131 - protein, 904 aa, Mus Musculus
MAWRCPRMGRVPLAWCLALCGWACMYPYDVPDYAAHKDTQTEAGSPFVGNPGNITGARGLTGTLRCELQVQGEPPEVVWLRDGQILELADNTQTQVPLGEDWQDEWKVVSQLRISALQLSDAGEYQCMVHLEGRTFVSQPGFVGLEGLPYFLEEPEDKAVPANTPFNLSCQAQGPPEPVTLLWLQDAVPLAPVTGHSSQHSLQTPGLNKTSSFSCEAHNAKGVTTSRTATITVLPQRPHHLHVVSRQPTELEVAWTPGLSGIYPLTHCNLQAVLSDDGVGIWLGKSDPPEDPLTLQVSVPPHQLRLEKLLPHTPYHIRISCSSSQGPSPWTHWLPVETTEGVPLGPPENVSAMRNGSQVLVRWQEPRVPLQGTLLGYRLAYRGQDTPEVLMDIGLTREVTLELRGDRPVANLTVSVTAYTSAGDGPWSLPVPLEPWRPGQGQPLHHLVSEPPPRAFSWPWWYVLLGAVVAAACVLILALFLVHRRKKETRYGEVFEPTVERGELVVRYRVRKSYSRRTTEATLNSLGISEELKEKLRDVMVDRHKVALGKTLGEGEFGAVMEGQLNQDDSILKVAVKTMKIAICTRSELEDFLSEAVCMKEFDHPNVMRLIGVCFQGSERESFPAPVVILPFMKHGDLHSFLLYSRLGDQPVYLPTQMLVKFMADIASGMEYLSTKRFIHRDLAARNCMLNENMSVCVADFGLSKKIYNGDYYRQGRIAKMPVKWIAIESLADRVYTSKSDVWSFGVTMWEIATRGQTPYPGVENSEIYDYLRQGNRLKQPADCLDGLYALMSRCWELNPQDRPSFTELREDLENTLKALPPAQEPDEILYVNMDEGGGYPEPPGAAGGADPPTQPDPKDSCSCLTAAEVHPAGRYVLCPSTTPSPAQPADRGSPAAPGQEDGA

SEQ ID NO: 132 - protein, 894 aa, homo sapiens
MAWRCPRMGRVPLAWCLALCGWACMAPRGTQAEESPFVGNPGNITGARGLTGTLRCQLQVQGEPPEVHWLRDGQILELADSTQTQVPLGEDEQDDWIVVSQLRITSLQLSDTGQYQCLVFLGHQTFVSQPGYVGLEGLPYFLEEPEDKAVPANTPFNLSCQAQGPPEPVTLLWLQDAVPLAPVTGHSSQHSLQTPGLNKTSSFSCEAHNAKGVTTSRTATITVLPQQPRNLHLVSRQPTELEVAWTPGLSGIYPLTHCTLQAVLSDDGMGIQAGEPDPPEEPLTSQASVPPHQLRLGSLHPHTPYHIRVACTSSQGPSSWTHWLPVETPEGVPLGPPENISATRNGSQAFVHWQEPRAPLQGTLLGYRLAYQGQDTPEVLMDIGLRQEVTLELQGDGSVSNLTVCVAAYTAAGDGPWSLPVPLEAWRPGQAQPVHQLVKEPSTPAFSWPWWYVLLGAVVAAACVLILALFLVHRRKKETRYGEVFEPTVERGELVVRYRVRKSYSRRTTEATLNSLGISEELKEKLRDVMVDRHKVALGKTLGEGEFGAVMEGQLNQDDSILKVAVKTMKIAICTRSELEDFLSEAVCMKEFDHPNVMRLIGVCFQGSERESFPAPVVILPFMKHGDLHSFLLYSRLGDQPVYLPTQMLVKFMADIASGMEYLSTKRFIHRDLAARNCMLNENMSVCVADFGLSKKIYNGDYYRQGRIAKMPVKWIAIESLADRVYTSKSDVWSFGVTMWEIATRGQTPYPGVENSEIYDYLRQGNRLKQPADCLDGLYALMSRCWELNPQDRPSFTELREDLENTLKALPPAQEPDEILYVNMDEGGGYPEPPGAAGGADPPTQPDPKDSCSCLTAAEVHPAGRYVLCPSTTPSPAQPADRGSPAAPGQEDGA

SEQ ID NO: 133 - protein, 894 aa, homo sapiens; identical to SEQ ID NO: 132

SEQ ID NO: 134 - protein, 894 aa, homo sapiens
MAWRCPRMGRVPLAWCLALCGWACMAPRGTQAEESPFVGNPGNITGARGLTGTLRCQLQVQGEPPEVHWLRDGQILELADSTQTQVPLGEDEQDDWIVVSQLRITSLQLSDTGQYQCLVFLGHQTFVSQPGYVGLEGLPYFLEEPEDRTVAANTPFNLSCQAQGPPEPVDLLWLQDAVPLATAPGHGPQRSLHVPGLNKTSSFSCEAHNAKGVTTSRTATITVLPQRPHHLHVVSRQPTELEVAWTPGLSGIYPLTHCNLQAVLSDDGVGIWLGKSDPPEDPLTLQVSVPPHQLRLEKLLPHTPYHIRISCSSSQGPSPWTHWLPVETTEGVPLGPPENISATRNGSQAFVHWQEPRAPLQGTLLGYRLAYQGQDTPEVLMDIGLRQEVTLELQGDGSVSNLTVCVAAYTAAGDGPWSLPVPLEAWRPGQAQPVHQLVKEPSTPAFSWPWWYVLLGAVVAAACVLILALFLVHRRKKETRYGEVFEPTVERGELVVRYRVRKSYSRRTTEATLNSLGISEELKEKLRDVMVDRHKVALGKTLGEGEFGAVMEGQLNQDDSILKVAVKTMKIAICTRSELEDFLSEAVCMKEFDHPNVMRLIGVCFQGSERESFPAPVVILPFMKHGDLHSFLLYSRLGDQPVYLPTQMLVKFMADIASGMEYLSTKRFIHRDLAARNCMLNENMSVCVADFGLSKKIYNGDYYRQGRIAKMPVKWIAIESLADRVYTSKSDVWSFGVTMWEIATRGQTPYPGVENSEIYDYLRQGNRLKQPADCLDGLYALMSRCWELNPQDRPSFTELREDLENTLKALPPAQEPDEILYVNMDEGGGYPEPPGAAGGADPPTQPDPKDSCSCLTAAEVHPAGRYVLCPSTTPSPAQPADRGSPAAPGQEDGA

SEQ ID NO: 135 - protein, 894 aa, homo sapiens
MAWRCPRMGRVPLAWCLALCGWACMAPRGTQAEESPFVGNPGNITGARGLTGTLRCQLQVQGEPPEVHWLRDGQILELADSTQTQVPLGEDEQDDWIVVSQLRITSLQLSDTGQYQCLVFLGHQTFVSQPGYVGLEGLPYFLEEPEDRTVAANTPFNLSCQAQGPPEPVDLLWLQDAVPLATAPGHGPQRSLHVPGLNKTSSFSCEAHNAKGVTTSRTATITVLPQQPRNLHLVSRQPTELEVAWTPGLSGIYPLTHCTLQAVLSDDGMGIQAGEPDPPEEPLTSQASVPPHQLRLGSLHPHTPYHIRVACTSSQGPSSWTHWLPVETPEGVPLGPPENVSAMRNGSQVLVRWQEPRVPLQGTLLGYRLAYRGQDTPEVLMDIGLTREVTLELRGDRPVANLTVSVTAYTSAGDGPWSLPVPLEPWRPGQGQPLHHLVSEPPPRAFSWPWWYVLLGAVVAAACVLILALFLVHRRKKETRYGEVFEPTVERGELVVRYRVRKSYSRRTTEATLNSLGISEELKEKLRDVMVDRHKVALGKTLGEGEFGAVMEGQLNQDDSILKVAVKTMKIAICTRSELEDFLSEAVCMKEFDHPNVMRLIGVCFQGSERESFPAPVVILPFMKHGDLHSFLLYSRLGDQPVYLPTQMLVKFMADIASGMEYLSTKRFIHRDLAARNCMLNENMSVCVADFGLSKKIYNGDYYRQGRIAKMPVKWIAIESLADRVYTSKSDVWSFGVTMWEIATRGQTPYPGVENSEIYDYLRQGNRLKQPADCLDGLYALMSRCWELNPQDRPSFTELREDLENTLKALPPAQEPDEILYVNMDEGGGYPEPPGAAGGADPPTQPDPKDSCSCLTAAEVHPAGRYVLCPSTTPSPAQPADRGSPAAPGQEDGA

SEQ ID NO: 136 - protein, 124 aa, homo sapiens
EVQLLESGGGLVQPGGSLRLSCAASGFTFSSYAMNWVRQAPGKGLEWVSGISGSGGHTYHADSVKGRFTISRDNSKNTLYLQMNSLRAEDTAVYYCAKDRYDILTGYYNLLDYWGQGTLVTVSS

SEQ ID NO: 137 - protein, 8 aa, homo sapiens
GFTFSSYA

SEQ ID NO: 138 - protein, 8 aa, homo sapiens
ISGSGGHT

SEQ ID NO: 139 - protein, 17 aa, homo sapiens
AKDRYDILTGYYNLLDY

SEQ ID NO: 140 - protein, 107 aa, homo sapiens
DIQMTQSPSSLSASVGDRVTITCRASQGISSWLAWYQQKPEEAPKSLIYAASSLQSGVPSRFSGSGSGTDFTLTISSLQPEDFATYYCQQYNSYPLTFGGGAKVEIK

SEQ ID NO: 141 - protein, 6 aa, homo sapiens
QGISSW

SEQ ID NO: 142 - protein, 9 aa, homo sapiens
QQYNSYPLT

SEQ ID NO: 143 - protein, 123 aa, homo sapiens
QVQLVQSGAEVKKPGASVKVSCKASGYAFTGYGISWVRQAPGQGLEWIGWISAYNGNTNYVQNLQDRVTMTTDTSTSTAYMELRSLRSDDTAVYYCARDHISMLRGIIIRNYWGQGTLVTVSS

SEQ ID NO: 144 - protein, 108 aa, homo sapiens
EIVLTQSPATLSLSPGERATLSCRASQSVSSYLAWYQQKPGQAPRLLIYDASNRATGIPARFSGSGSGTDFTLTISSLEPEDFAVYYCQQRSSWPRLTFGGGTKVEIK

SEQ ID NO: 145 - protein, 124 aa, homo sapiens
QVQLVQSGAEVKKPGSSVKVSCKASGGTFSRYAISWVRQAPGQGLEWMGRIIPIVGIANYAQKFQGRVTLTADKSTSTAYMELSSLRSEDTAVYYCAREAGYSSSWYAEYFQHWGQGTLVTVSS

SEQ ID NO: 146 - protein, 108 aa, homo sapiens
EIVLTQSPGTLSLSPGERATLSCRASQSVSSNYLAWYQQKPGQAPRLLIYGASSRATGFPDRFSGSGSGTDFTLTISRLEPEDFAVYYCQQYGSSPYTFGQGTKLEIK

SEQ ID NO: 147 - protein, 893 aa, Macaca fascicularis
AWRCPRMGRVPLAWCLALCGWVCMAPRGTQAEESPFVGNPGNITGARGLTGTLRCQLQVQGEPPEVHWLRDGQILELADSTQTQVPLGEDEQDDWIVVSQLRIASLQLSDAGQYQCLVFLGHQNFVSQPGYVGLEGLPYFLEEPEDRTVAANTPFNLSCQAQGPPEPVDLLWLQDAVPLATAPGHGPQRNLHVPGLNKTSSFSCEAHNAKGVTTSRTATITVLPQQPRNLHLVSRQPTELEVAWTPGLSGIYPLTHCTLQAVLSDDGMGIQAGEPDPPEEPLTLQASVPPHQLRLGSLHPHTPYHIRVACTSSQGPSSWTHWLPVETPEGVPLGPPENISATRNGSQAFVHWQEPRAPLQGTLLGYRLAYQGQDTPEVLMDIGLRQEVTLELQGDGSVSNLTVCVAAYTAAGDGPWSLPVPLEAWRPGQAQPVHQLVKETSAPAFSWPWWYILLGAVVAAACVLILALFLVHRRKKETRYGEVFEPTVERGELVVRYRVRKSYSRRTTEATLNSLGISEELKEKLRDVMVDRHKVALGKTLGEGEFGAVMEGQLNQDDSILKVAVKTMKIAICTRSELEDFLSEAVCMKEFDHPNVMRLIGVCFQGSERESFPAPVVILPFMKHGDLHSFLLYSRLGDQPVYLPTQMLVKFMADIASGMEYLSTKRFIHRDLAARNCMLNENMSVCVADFGLSKKIYNGDYYRQGRIAKMPVKWIAIESLADRVYTSKSDVWSFGVTMWEIATRGQTPYPGVENSEIYDYLRQGNRLKQPADCLDGLYALMSRCWELNPQDRPSFTELREDLENTLKALPPAQEPDEILYVNMDEGGGYPEPPGAAGGADPPTQLDPKDSCSCLTSAEVHPAGRYVLCPSTAPSPAQPADRGSPAAPGQEDGA

SEQ ID NO: 148 - protein, 903 aa, Homo sapiens
MAWRCPRMGRVPLAWCLALCGWACMYPYDVPDYAAPRGTQAEESPFVGNPGNITGARGLTGTLRCQLQVQGEPPEVHWLRDGQILELADSTQTQVPLGEDEQDDWIVVSQLRITSLQLSDTGQYQCLVFLGHQTFVSQPGYVGLEGLPYFLEEPEDRTVAANTPFNLSCQAQGPPEPVDLLWLQDAVPLATAPGHGPQRSLHVPGLNKTSSFSCEAHNAKGVTTSRTATITVLPQQPRNLHLVSRQPTELEVAWTPGLSGIYPLTHCTLQAVLSNDGMGIQAGEPDPPEEPLTSQASVPPHQLRLGSLHPHTPYHIRVACTSSQGPSSWTHWLPVETPEGVPLGPPENISATRNGSQAFVHWQEPRAPLQGTLLGYRLAYQGQDTPEVLMDIGLRQEVTLELQGDGSVSNLTVCVAAYTAAGDGPWSLPVPLEAWRPGQAQPVHQLVKEPSTPAFSWPWWYVLLGAVVAAACVLILALFLVHRRKKETRYGEVFEPTVERGELVVRYRVRKSYSRRTTEATLNSLGISEELKEKLRDVMVDRHKVALGKTLGEGEFGAVMEGQLNQDDSILKVAVKTMKIAICTRSELEDFLSEAVCMKEFDHPNVMRLIGVCFQGSERESFPAPVVILPFMKHGDLHSFLLYSRLGDQPVYLPTQMLVKFMADIASGMEYLSTKRFIHRDLAARNCMLNENMSVCVADFGLSKKIYNGDYYRQGRIAKMPVKWIAIESLADRVYTSKSDVWSFGVTMWEIATRGQTPYPGVENSEIYDYLRQGNRLKQPADCLDGLYALMSRCWELNPQDRPSFTELREDLENTLKALPPAQEPDEILYVNMDEGGGYPEPPGAAGGADPPTQPDPKDSCSCLTAAEVHPAGRYVLCPSTTPSPAQPADRGSPAAPGQEDGA

SEQ ID NO: 149 - protein, 904 aa, Mus musculus; identical to SEQ ID NO: 131

SEQ ID NO: 150 - protein, 888 aa, Mus musculus
MGRVPLAWWLALCCWGCAAHKDTQTEAGSPFVGNPGNITGARGLTGTLRCELQVQGEPPEVVWLRDGQILELADNTQTQVPLGEDWQDEWKVVSQLRISALQLSDAGEYQCMVHLEGRTFVSQPGFVGLEGLPYFLEEPEDRTVAANTPFNLSCQAQGPPEPVDLLWLQDAVPLATAPGHGPQRSLHVPGLNKTSSFSCEAHNAKGVTTSRTATITVLPQQPRNLHLVSRQPTELEVAWTPGLSGIYPLTHCTLQAVLSDDGMGIQAGEPDPPEEPLTSQASVPPHQLRLGSLHPHTPYHIRVACTSSQGPSSWTHWLPVETPEGVPLGPPENISATRNGSQAFVHWQEPRAPLQGTLLGYRLAYQGQDTPEVLMDIGLRQEVTLELQGDGSVSNLTVCVAAYTAAGDGPWSLPVPLEAWRPGQAQPVHQLVKEPSTPAFSWPWWYVLLGAVVAAACVLILALFLVHRRKKETRYGEVFEPTVERGELVVRYRVRKSYSRRTTEATLNSLGISEELKEKLRDVMVDRHKVALGKTLGEGEFGAVMEGQLNQDDSILKVAVKTMKIAICTRSELEDFLSEAVCMKEFDHPNVMRLIGVCFQGSERESFPAPVVILPFMKHGDLHSFLLYSRLGDQPVYLPTQMLVKFMADIASGMEYLSTKRFIHRDLAARNCMLNENMSVCVADFGLSKKIYNGDYYRQGRIAKMPVKWIAIESLADRVYTSKSDVWSFGVTMWEIATRGQTPYPGVENSEIYDYLRQGNRLKQPADCLDGLYALMSRCWELNPQDRPSFTELREDLENTLKALPPAQEPDEILYVNMDEGGGYPEPPGAAGGADPPTQPDPKDSCSCLTAAEVHPAGRYVLCPSTTPSPAQPADRGSPAAPGQEDGA

SEQ ID NO: 151 - protein, 894 aa, Artificial; identical to SEQ ID NO: 132
  Chimeric protein construct

SEQ ID NO: 152 - protein, 894 aa, Artificial; identical to SEQ ID NO: 134
  Chimeric protein construct

SEQ ID NO: 153 - protein, 894 aa, Artificial; identical to SEQ ID NO: 135
  Chimeric protein construct